European Patent Application EP 4 814 133 A1, published September 30, 2026. Title: 快速检测分枝杆菌的方法. Applicant: 上海科技大学. The sequence listing filed with the application follows.

SEQUENCE LISTING (32 sequences)

SEQ ID NO: 1 - DNA, 50 bp, synthetic construct
  source 1..50: mol_type = other DNA
aattctaatacgactcactataggggccggctacccgtcgtcgccttggt

SEQ ID NO: 2 - DNA, 51 bp, synthetic construct
  source 1..51: mol_type = other DNA
aattctaatacgactcactatagggccctctcaggccggctacccgtcgtc

SEQ ID NO: 3 - DNA, 20 bp, synthetic construct
  source 1..20: mol_type = other DNA
taacacatgcaagtcgaacg

SEQ ID NO: 4 - DNA, 20 bp, synthetic construct
  source 1..20: mol_type = other DNA
cgagtggcgaacgggtgagt

SEQ ID NO: 5 - DNA, 22 bp, synthetic construct
  source 1..22: mol_type = other DNA
gataagcctgggaaactgggtc

SEQ ID NO: 6 - DNA, 21 bp, synthetic construct
  source 1..21: mol_type = other DNA
ctgggaaactgggtctaatac

SEQ ID NO: 7 - RNA, 23 nt, synthetic construct
  source 1..23: mol_type = other RNA
ccagcggataggaccacggctgg

SEQ ID NO: 8 - DNA, 25 bp, synthetic construct
  source 1..25: mol_type = other DNA
gaaattaatacgactcactataggg

SEQ ID NO: 9 - RNA, 67 nt, synthetic construct
  source 1..67: mol_type = other RNA
ggggatttagactaccccaaaaacgaaggggactaaaaccttgtggtggaaagcgctttagcggtgt

SEQ ID NO: 10 - RNA, 67 nt, synthetic construct
  source 1..67: mol_type = other RNA
ggggatttagactaccccaaaaacgaaggggactaaaaccatgtcttgtggtggaaagcgctttagc

SEQ ID NO: 11 - RNA, 67 nt, synthetic construct
  source 1..67: mol_type = other RNA
ggggatttagactaccccaaaaacgaaggggactaaaacggtggaaagcgctttagcggtgtgggat

SEQ ID NO: 12 - RNA, 67 nt, synthetic construct
  source 1..67: mol_type = other RNA
ggggatttagactaccccaaaaacgaaggggactaaaaccgggatgcatgtcttgtggtggaaagcg

SEQ ID NO: 13 - RNA, 67 nt, synthetic construct
  source 1..67: mol_type = other RNA
ggggatttagactaccccaaaaacgaaggggactaaaacgataggaccacgggatgcatgtcttggg

SEQ ID NO: 14 - RNA, 67 nt, synthetic construct
  source 1..67: mol_type = other RNA
ggggatttagactaccccaaaaacgaaggggactaaaacaccggataggaccacgggatgcatgtct

SEQ ID NO: 15 - RNA, 67 nt, synthetic construct
  source 1..67: mol_type = other RNA
ggggatttagactaccccaaaaacgaaggggactaaaacgcccgcggcctatcagcttgttggtggg

SEQ ID NO: 16 - RNA, 67 nt, synthetic construct
  source 1..67: mol_type = other RNA
ggggatttagactaccccaaaaacgaaggggactaaaacaataggaccacaggacacatgtcctgtg

SEQ ID NO: 17 - RNA, 67 nt, synthetic construct
  source 1..67: mol_type = other RNA
ggggatttagactaccccaaaaacgaaggggactaaaacgataggaccacacacttcatggtgagtg

SEQ ID NO: 18 - RNA, 67 nt, synthetic construct
  source 1..67: mol_type = other RNA
ggggatttagactaccccaaaaacgaaggggactaaaacaatatgaccacgcgcttcatggtgtgtg

SEQ ID NO: 19 - RNA, 67 nt, synthetic construct
  source 1..67: mol_type = other RNA
ggggatttagactaccccaaaaacgaaggggactaaaacgataggacctcaagacgcatgtcttctg

SEQ ID NO: 20 - RNA, 67 nt, synthetic construct
  source 1..67: mol_type = other RNA
ggggatttagactaccccaaaaacgaaggggactaaaacgataggacctttaggcgcatgtctttag

SEQ ID NO: 21 - RNA, 67 nt, synthetic construct
  source 1..67: mol_type = other RNA
ggggatttagactaccccaaaaacgaaggggactaaaacgataggaccacttggcgcatgccttgtg

SEQ ID NO: 22 - protein, 1184 aa, Leptotrichia wadei
MGSSHHHHHHSSGLVPRGSMKVTKVDGISHKKYIEEGKLVKSTSEENRTSERLSELLSIRLDIYIKNPDNASEEENRIRRENLKKFFSNKVLHLKDSVLYLKNRKEKNAVQDKNYSEEDISEYDLKNKNSFSVLKKILLNEDVNSEELEIFRKDVEAKLNKINSLKYSFEENKANYQKINENNVEKVGGKSKRNIIYDYYRESAKRNDYINNVQEAFDKLYKKEDIEKLFFLIENSKKHEKYKIREYYHKIIGRKNDKENFAKIIYEEIQNVNNIKELIEKIPDMSELKKSQVFYKYYLDKEELNDKNIKYAFCHFVEIEMSQLLKNYVYKRLSNISNDKIKRIFEYQNLKKLIENKLLNKLDTYVRNCGKYNYYLQVGEIATSDFIARNRQNEAFLRNIIGVSSVAYFSLRNILETENENDITGRMRGKTVKNNKGEEKYVSGEVDKIYNENKQNEVKENLKMFYSYDFNMDNKNEIEDFFANIDEAISSIRHGIVHFNLELEGKDIFAFKNIAPSEISKKMFQNEINEKKLKLKIFKQLNSANVFNYYEKDVIIKYLKNTKFNFVNKNIPFVPSFTKLYNKIEDLRNTLKFFWSVPKDKEEKDAQIYLLKNIYYGEFLNKFVKNSKVFFKITNEVIKINKQRNQKTGHYKYQKFENIEKTVPVEYLAIIQSREMINNQDKEEKNTYIDFIQQIFLKGFIDYLNKNNLKYIESNNNNDNNDIFSKIKIKKDNKEKYDKILKNYEKHNRNKEIPHEINEFVREIKLGKILKYTENLNMFYLILKLLNHKELTNLKGSLEKYQSANKEETFSDELELINLLNLDNNRVTEDFELEANEIGKFLDFNENKIKDRKELKKFDTNKIYFDGENIIKHRAFYNIKKYGMLNLLEKIADKAKYKISLKELKEYSNKKNEIEKNYTMQQNLHRKYARPKKDEKFNDEDYKEYEKAIGNIQKYTHLKNKVEFNELNLLQGLLLKILHRLVGYTSIWERDLRFRLKGEFPENHYIEEIFNFDNSKNVKYKSGQIVEKYINFYKELYKDNVEKRSIYSDKKVKKLKQEKKDLYIRNYIAHFNYIPHAEISLLEVLENLRKLLSYDRKLKNAIMKSIVDILKEYGFVATFKIGADKKIEIQTLESEKIVHLKNLKKKKLMTDRNSEELCELVKVMFEYKALEKLAAALEHHHHHH

SEQ ID NO: 23 - DNA, 3498 bp, synthetic construct
  source 1..3498: mol_type = other DNA
atgaaagtgaccaaggtcgacggcatcagccacaagaagtacatcgaagagggcaagctcgtgaagtccaccagcgaggaaaaccggaccagcgagagactgagcgagctgctgagcatccggctggacatctacatcaagaaccccgacaacgcctccgaggaagagaaccggatcagaagagagaacctgaagaagttctttagcaacaaggtgctgcacctgaaggacagcgtgctgtatctgaagaaccggaaagaaaagaacgccgtgcaggacaagaactatagcgaagaggacatcagcgagtacgacctgaaaaacaagaacagcttctccgtgctgaagaagatcctgctgaacgaggacgtgaactctgaggaactggaaatctttcggaaggacgtggaagccaagctgaacaagatcaacagcctgaagtacagcttcgaagagaacaaggccaactaccagaagatcaacgagaacaacgtggaaaaagtgggcggcaagagcaagcggaacatcatctacgactactacagagagagcgccaagcgcaacgactacatcaacaacgtgcaggaagccttcgacaagctgtataagaaagaggatatcgagaaactgtttttcctgatcgagaacagcaagaagcacgagaagtacaagatccgcgagtactatcacaagatcatcggccggaagaacgacaaagagaacttcgccaagattatctacgaagagatccagaacgtgaacaacatcaaagagctgattgagaagatccccgacatgtctgagctgaagaaaagccaggtgttctacaagtactacctggacaaagaggaactgaacgacaagaatattaagtacgccttctgccacttcgtggaaatcgagatgtcccagctgctgaaaaactacgtgtacaagcggctgagcaacatcagcaacgataagatcaagcggatcttcgagtaccagaatctgaaaaagctgatcgaaaacaaactgctgaacaagctggacacctacgtgcggaactgcggcaagtacaactactatctgcaagtgggcgagatcgccacctccgactttatcgcccggaaccggcagaacgaggccttcctgagaaacatcatcggcgtgtccagcgtggcctacttcagcctgaggaacatcctggaaaccgagaacgagaacgatatcaccggccggatgcggggcaagaccgtgaagaacaacaagggcgaagagaaatacgtgtccggcgaggtggacaagatctacaatgagaacaagcagaacgaagtgaaagaaaatctgaagatgttctacagctacgacttcaacatggacaacaagaacgagatcgaggacttcttcgccaacatcgacgaggccatcagcagcatcagacacggcatcgtgcacttcaacctggaactggaaggcaaggacatcttcgccttcaagaatatcgcccccagcgagatctccaagaagatgtttcagaacgaaatcaacgaaaagaagctgaagctgaaaatcttcaagcagctgaacagcgccaacgtgttcaactactacgagaaggatgtgatcatcaagtacctgaagaataccaagttcaacttcgtgaacaaaaacatccccttcgtgcccagcttcaccaagctgtacaacaagattgaggacctgcggaataccctgaagtttttttggagcgtgcccaaggacaaagaagagaaggacgcccagatctacctgctgaagaatatctactacggcgagttcctgaacaagttcgtgaaaaactccaaggtgttctttaagatcaccaatgaagtgatcaagattaacaagcagcggaaccagaaaaccggccactacaagtatcagaagttcgagaacatcgagaaaaccgtgcccgtggaatacctggccatcatccagagcagagagatgatcaacaaccaggacaaagaggaaaagaatacctacatcgactttattcagcagattttcctgaagggcttcatcgactacctgaacaagaacaatctgaagtatatcgagagcaacaacaacaatgacaacaacgacatcttctccaagatcaagatcaaaaaggataacaaagagaagtacgacaagatcctgaagaactatgagaagcacaatcggaacaaagaaatccctcacgagatcaatgagttcgtgcgcgagatcaagctggggaagattctgaagtacaccgagaatctgaacatgttttacctgatcctgaagctgctgaaccacaaagagctgaccaacctgaagggcagcctggaaaagtaccagtccgccaacaaagaagaaaccttcagcgacgagctggaactgatcaacctgctgaacctggacaacaacagagtgaccgaggacttcgagctggaagccaacgagatcggcaagttcctggacttcaacgaaaacaaaatcaaggaccggaaagagctgaaaaagttcgacaccaacaagatctatttcgacggcgagaacatcatcaagcaccgggccttctacaatatcaagaaatacggcatgctgaatctgctggaaaagatcgccgataaggccaagtataagatcagcctgaaagaactgaaagagtacagcaacaagaagaatgagattgaaaagaactacaccatgcagcagaacctgcaccggaagtacgccagacccaagaaggacgaaaagttcaacgacgaggactacaaagagtatgagaaggccatcggcaacatccagaagtacacccacctgaagaacaaggtggaattcaatgagctgaacctgctgcagggcctgctgctgaagatcctgcaccggctcgtgggctacaccagcatctgggagcgggacctgagattccggctgaagggcgagtttcccgagaaccactacatcgaggaaattttcaatttcgacaactccaagaatgtgaagtacaaaagcggccagatcgtggaaaagtatatcaacttctacaaagaactgtacaaggacaatgtggaaaagcggagcatctactccgacaagaaagtgaagaaactgaagcaggaaaaaaaggacctgtacatccggaactacattgcccacttcaactacatcccccacgccgagattagcctgctggaagtgctggaaaacctgcggaagctgctgtcctacgaccggaagctgaagaacgccatcatgaagtccatcgtggacattctgaaagaatacggcttcgtggccaccttcaagatcggcgctgacaagaagatcgaaatccagaccctggaatcagagaagatcgtgcacctgaagaatctgaagaaaaagaaactgatgaccgaccggaacagcgaggaactgtgcgaactcgtgaaagtcatgttcgagtacaaggccctggaaaagcttgcggccgcactcgagcaccaccaccaccaccactga

SEQ ID NO: 24 - DNA, 20 bp, synthetic construct
  source 1..20: mol_type = other DNA
taatacgactcactataggg

SEQ ID NO: 25 - DNA, 342 bp, synthetic construct
  source 1..342: mol_type = other DNA
ttttgtttggagagtttgatcctggctcaggacgaacgctggcggcgtgcttaacacatgcaagtcgaacggaaaggtctcttcggagatactcgagtggcgaacgggtgagtaacacgtgggtgatctgccctgcacttcgggataagcctgggaaactgggtctaataccggataggaccacgggatgcatgtcttgtggtggaaagcgctttagcggtgtgggatgagcccgcggcctatcagcttgttggtggggtgacggcctaccaaggcgacgacgggtagccggcctgagagggtgtccggccacactgggactgagatacggcccagactcct

SEQ ID NO: 26 - DNA, 338 bp, synthetic construct
  source 1..338: mol_type = other DNA
ttttgtttggagagtttgatcctggctcaggacgaacgctggcggcgtgcttaacacatgcaagtcgaacggaaaggcccttcggggtactcgagtggcgaacgggtgagtaacacgtgggtgatctgccctgcactctgggataagcctgggaaactgggtctaataccggataggaccacacacttcatggtgagtggtgcaaagcttttgcggtgtgggatgagcccgcggcctatcagcttgttggtggggtaatggcccaccaaggcgacgacgggtagccggcctgagagggtgaccggccacactgggactgagatacggcccagactcct

SEQ ID NO: 27 - DNA, 330 bp, synthetic construct
  source 1..330: mol_type = other DNA
agagtttgatcctggctcaggacgaacgctggcggcgtgcttaacacatgcaagtcgaacggaaaggcctcttcggaggtactcgagtggcgaacgggtgagtaacacgtgggcaatctgccctgcacttcgggataagcctgggaaactgggtctaataccggataggacctcaagacgcatgtcttctggtggaaagcttttgcggtgtgggatgggcccgcggcctatcagcttgttggtggggtgacggcctaccaaggcgacgacgggtagccggcctgagagggtgtccggccacactgggactgagatacggcccagactcct

SEQ ID NO: 28 - DNA, 328 bp, synthetic construct
  source 1..328: mol_type = other DNA
agagtttgatcctggctcaggacgaacgctggcggcgtgcttaacacatgcaagtcgaacggaaaggcccttcggggtactcgagtggcgaacgggtgagtaacacgtgggtgatctgccctgcactttgggataagcctgggaaactgggtctaataccgaatatgaccacgcgcttcatggtgtgtggtggaaagcttttgcggtgtgggatgggcccgcggcctatcagcttgttggtggggtaatggcctaccaaggcgacgacgggtagccggcctgagagggtgaccggccacactgggactgagatacggcccagactcct

SEQ ID NO: 29 - DNA, 308 bp, synthetic construct
  source 1..308: mol_type = other DNA
gacgaacgctggcggcgtgcttaacacatgcaagtcgaacggtaaggcccttcggggtacacgagtggcgaacgggtgagtaacacgtgggtaatctgccctgcacatcgggataagcctgggaaactgggtctaataccgaataggaccacaggacacatgtcctgtggtggaaagcttttgcggtgtgggatgggcccgcggcctatcagcttgttggtggggtgatggcctaccaaggcgacgacgggtagccggcctgagagggtgtccggccacactgggactgagatacggcccagactcct

SEQ ID NO: 30 - DNA, 330 bp, synthetic construct
  source 1..330: mol_type = other DNA
agagtttgatcctggctcaggacgaacgctggcggcgtgcttaacacatgcaagtcgaacggaaaggccccttcgggggtactcgagtggcgaacgggtgagtaacacgtgggcaatctgccctgcacttcgggataagcctgggaaactgggtctaataccggataggacctttaggcgcatgtctttaggtggaaagcttttgcggtgtgggatgggcccgcggcctatcagcttgttggtggggtgatggcctaccaaggcgacgacgggtagccggcctgagagggtgtccggccacactgggactgagatacggcccagactcct

SEQ ID NO: 31 - DNA, 337 bp, synthetic construct
  source 1..337: mol_type = other DNA
tgtttggagagtttgatcctggctcaggacgaacgctggcggcgtgcttaacacatgcaagtcgaacggaaaggtctcttcggagacactcgagtggcgaacgggtgagtaacacgtgggcaatctgccctgcacaccgggataagcctgggaaactgggtctaataccggataggaccacttggcgcatgccttgtggtggaaagcttttgcggtgtgggatgggcccgcggcctatcagcttgttggtggggtgacggcctaccaaggcgacgacgggtagccggcctgagagggtgtccggccacactgggactgagatacggcccagactcct

SEQ ID NO: 32 - DNA, 302 bp, synthetic construct
  source 1..302: mol_type = other DNA
agagtttgatcctggctcaggacgaacgctggcggcgtgcttaacacatgcaagtcgaacggaaaggctggtactcgagtggcgaacgggtgagtaacacgtgggatctgccctgcacgggataagcctgggaaactgggtctaataccgataggacccgcatgttggtggaaagcttttgcggtgtgggatggcccgcggcctatcagcttgttggtggggtaggcctaccaaggcgacgacgggtagccggcctgagagggtgccggccacactgggactgagatacggcccagactcct